European Patent Specification EP 3 259 345 B1, published February 8, 2023. Title: USE OF A LAMININ FOR DIFFERENTIATING PLURIPOTENT CELLS INTO HEPATOCYTE LINEAGE CELLS. Applicant: NGuyen, Tuan huy INSERM. The sequence listing filed with the application follows.

SEQUENCE LISTING (20 sequences)

SEQ ID NO: 1 - DNA, 20 bp, Artificial Sequence
  source 1..20: /mol_type="unassigned DNA" /note="primer AFP-F" /organism="Artificial Sequence"
gcttggtggtggatgaaaca

SEQ ID NO: 2 - DNA, 23 bp, Artificial Sequence
  source 1..23: /mol_type="unassigned DNA" /note="AFP-R" /organism="Artificial Sequence"
tcctctgttatttgtggcttttg

SEQ ID NO: 3 - DNA, 22 bp, Artificial Sequence
  source 1..22: /mol_type="unassigned DNA" /note="ALB-F" /organism="Artificial Sequence"
gcacagaatccttggtgaacag

SEQ ID NO: 4 - DNA, 23 bp, Artificial Sequence
  source 1..23: /mol_type="unassigned DNA" /note="ALB-R" /organism="Artificial Sequence"
atggaaggtgaatgttttcagca

SEQ ID NO: 5 - DNA, 20 bp, Artificial Sequence
  source 1..20: /mol_type="unassigned DNA" /note="CK19-F" /organism="Artificial Sequence"
ctcccgcgactacagccact

SEQ ID NO: 6 - DNA, 20 bp, Artificial Sequence
  source 1..20: /mol_type="unassigned DNA" /note="CK19-R" /organism="Artificial Sequence"
tcagctcatccagcaccctg

SEQ ID NO: 7 - DNA, 22 bp, Artificial Sequence
  source 1..22: /mol_type="unassigned DNA" /note="CYP3A4-F" /organism="Artificial Sequence"
agatgcctttaggtccaatggg

SEQ ID NO: 8 - DNA, 21 bp, Artificial Sequence
  source 1..21: /mol_type="unassigned DNA" /note="CYP3A4-R" /organism="Artificial Sequence"
gctggagatagcaatgttcgt

SEQ ID NO: 9 - DNA, 20 bp, Artificial Sequence
  source 1..20: /mol_type="unassigned DNA" /note="CYP3A7-F" /organism="Artificial Sequence"
aaggtcgcctcaaagagaca

SEQ ID NO: 10 - DNA, 20 bp, Artificial Sequence
  source 1..20: /mol_type="unassigned DNA" /note="CYP3A7-R" /organism="Artificial Sequence"
tgcactttctgctggacatc

SEQ ID NO: 11 - DNA, 19 bp, Artificial Sequence
  source 1..19: /mol_type="unassigned DNA" /note="FOXA2-F" /organism="Artificial Sequence"
gcactcggcttccagtatg

SEQ ID NO: 12 - DNA, 20 bp, Artificial Sequence
  source 1..20: /mol_type="unassigned DNA" /note="FOXA2-R" /organism="Artificial Sequence"
cacgtacgacgacatgttca

SEQ ID NO: 13 - DNA, 20 bp, Artificial Sequence
  source 1..20: /mol_type="unassigned DNA" /note="GAPDH-F" /organism="Artificial Sequence"
aatcccatcaccatcttcca

SEQ ID NO: 14 - DNA, 20 bp, Artificial Sequence
  source 1..20: /mol_type="unassigned DNA" /note="GAPDH-R" /organism="Artificial Sequence"
tggactccacgacgtactca

SEQ ID NO: 15 - DNA, 21 bp, Artificial Sequence
  source 1..21: /mol_type="unassigned DNA" /note="HNF4-F" /organism="Artificial Sequence"
tggacaaagacaagaggaacc

SEQ ID NO: 16 - DNA, 20 bp, Artificial Sequence
  source 1..20: /mol_type="unassigned DNA" /note="HNF4-R" /organism="Artificial Sequence"
atagcttgaccttcgagtgc

SEQ ID NO: 17 - DNA, 20 bp, Artificial Sequence
  source 1..20: /mol_type="unassigned DNA" /note="SOX2-F" /organism="Artificial Sequence"
cctactcgcagcagggcacc

SEQ ID NO: 18 - DNA, 20 bp, Artificial Sequence
  source 1..20: /mol_type="unassigned DNA" /note="SOX2-R" /organism="Artificial Sequence"
ctcggcgccggggagataca

SEQ ID NO: 19 - DNA, 20 bp, Artificial Sequence
  source 1..20: /mol_type="unassigned DNA" /note="SOX17-F" /organism="Artificial Sequence"
tttcatggtgtgggctaagg

SEQ ID NO: 20 - DNA, 19 bp, Artificial Sequence
  source 1..19: /mol_type="unassigned DNA" /note="SOX17-R" /organism="Artificial Sequence"
cggccggtacttgtagttg